European Patent Application EP 4 154 908 A1, published March 29, 2023. Title: COMPOSITIONS AND METHODS FOR TREATING, INCLUDING PREVENTING, PARVOVIRUS INFECTIONS AND RELATED DISEASES. Applicant: University of Louisville Research Foundation, Inc. Application EP. The sequence listing filed with the application follows.

SEQUENCE LISTING (76 sequences)

SEQ ID NO: 1 - protein, 554 aa, Parvovirus B19
MTSVNSAEASTGAGGGGSNPVKSMWSEGATFSANSVTCTFSRQFLIPYDPEHHYKVFSPAASSCHNASGKEAKVCTISPIMGYSTPWRYLDFNALNLFFSPLEFQHLIENYGSIAPDALTVTISEIAVKDVTDKTGGGVQVTDSTTGRLCMLVDHEYKYPYVLGQGQDTLAPELPIWVYFPPQYAYLTVGDVNTQGISGDSKKLASEESAFYVLEHSSFQLLGTGGTATMSYKFPPVPPENLEGCSQHFYEMYNPLYGSRLGVPDTLGGDPKFRSLTHEDHAIQPQNFMPGPLVNSVSTKEGDSSNTGAGKALTGLSTGTSQNTRISLRPGPVSQPYHHWDTDKYVTGINAISHGQTTYGNAEDKEYQQGVGRFPNEKEQLKQLQGLNMHTYFPNKGTQQYTDQIERPLMVGSVWNRRALHYESQLWSKIPNLDDSFKTQFAALGGWGLHQPPPQIFLKILPQSGPIGGIKSMGITTLVQYAVGIMTVTMTFKLGPRKATGRWNPQPGVYPPHAAGHLPYVLYDPTATDAKQHHRHGYEKPEELWTAKSRVHPL

SEQ ID NO: 2 - DNA, 1665 bp, Parvovirus B19
  source 1..1665: mol_type = unassigned DNA
atgacttcagttaattctgcagaagccagcactggtgcaggaggggggggcagtaatcctgtcaaaagcatgtggagtgagggggccacttttagtgccaactctgtgacttgtacattttctagacagtttttaattccatatgacccagagcaccattataaggtgttttctcccgcagcaagtagctgccacaatgccagtggaaaggaggcaaaggtttgcaccattagtcccataatgggatactcaaccccatggagatatttagattttaatgctttaaacttatttttttcacctttagagtttcagcacttaattgaaaattatggaagtatagctcctgatgctttaactgtaaccatatcagaaattgctgttaaggatgttacagacaaaactggagggggggtgcaggttactgacagcactacagggcgcctatgcatgttagtagaccatgaatacaagtacccatatgtgttagggcaaggtcaagatactttagccccagaacttcctatttgggtatactttccccctcaatatgcttacttaacagtaggagatgttaacacacaaggaatttctggagacagcaaaaaattagcaagtgaagaatcagcattttatgttttggaacacagttcttttcagcttttaggtacaggaggtacagcaactatgtcttataagtttcctccagtgcccccagaaaatttagagggctgcagtcaacacttttatgagatgtacaatcccttatacggatcccgcttaggggttcctgacacattaggaggtgacccaaaatttagatctttaacacatgaagaccatgcaattcagccccaaaacttcatgccagggccactagtaaactcagtgtctacaaaggagggagacagctctaatactggagctgggaaagccttaacaggccttagcacaggtacctctcaaaacactagaatatccttacgcccggggccagtgtctcagccgtaccaccactgggacacagataaatatgtcacaggaataaatgctatttctcatggtcagaccacttatggtaacgctgaagacaaagagtatcagcaaggagtgggtagatttccaaatgaaaaagaacagctaaaacagttacagggtttaaacatgcacacctactttcccaataaaggaacccagcaatatacagatcaaattgagcgccccctaatggtgggttctgtatggaacagaagagcccttcactatgaaagccagctgtggagtaaaattccaaatttagatgacagttttaaaactcagtttgcagccttaggaggatggggtttgcatcagccacctcctcaaatatttttaaaaatattaccacaaagtgggccaattggaggtattaaatcaatgggaattactaccttagttcagtatgccgtgggaattatgacagtaaccatgacatttaaattggggccccgtaaagctacgggacggtggaatcctcaacctggagtatatcccccgcacgcagcaggtcatttaccatatgtactatatgaccctacagctacagatgcaaaacaacaccacagacatggatatgaaaagcctgaagaattgtggacagccaaaagccgtgtgcacccattgtaa

SEQ ID NO: 3 - DNA, 1665 bp, synthetic construct
  misc_feature 1..1665: note = Construct A
  source 1..1665: mol_type = other DNA
atgacttcagttaattctgcagaagccagcactggtgcaggaggggggggcagtaatcctgtcaaaagcatgtggagtgagggggccacttttagtgccaactctgtgacttgtacattttctagacagtttttaattccatatgacccagagcaccattataaggtgttttctcccgcagcaagtagctgccacaatgccagtggaaaggaggcaaaggtttgcaccattagtcccataatgggatactcaaccccatggagatatttagattttaatgctttaaacttatttttttcacctttagagtttcagcacttaattgaaaattatggaagtatagctcctgatgctttaactgtaaccatatcagaaattgctgttaaggatgttacagacaaaactggagggggggtgcaggttactgacagcactacagggcgcctatgcatgttagtagaccatgaatacaagtacccatatgtgttagggcaaggtcaagatactttagccccagaacttcctatttgggtatactttccccctcaatatgcttacttaacagtaggagatgttaacacacaaggaatttctggagacagcaaaaaattagcaagtgaagaatcagcattttatgttttggaacacagttcttttcagcttttaggtacaggaggtacagcaactatgtcttataagtttcctccagtgcccccagaaaatttagagggctgcagtcaacacttttatgagatgtacaatcccttatacggatcccgcttaggggttcctgacacattaggaggtgacccaaaatttagatctttaacacatgaagaccatgcaattcagccccaaaacttcatgccagggccactagtaaactcagtgtctacaaaggagggagacagctctaatactggagctgggaaagccttaacaggccttagcacaggtacctctcaaaacactagaatatccttacgcccggggccagtgtctcagccgtaccaccactgggacacagataaatatgtcacaggaataaatgctatttctcatggtcagaccacttatggtaacgctgaagacaaagagtatcagcaaggagtgggtagatttccaaatgaaaaagaacagctaaaacagttacagggtttaaacatgcacacctactttcccaataaaggaacccagcaatttacagatcaaattgagcgccccctaatggtgggttctgtatggaacagaagagcccttcactatgaaagccagctgtggagtaaaattccaaatttagatgacagttttaaaactcagtttgcagccttaggaggatggggtttgcatcagccacctcctcaaatatttttaaaaatattaccacaaagtgggccaattggaggtattaaatcaatgggaattactaccttagttcagtatgccgtgggaattatgacagtaaccatgacatttaaattggggccccgtaaagctacgggacggtggaatcctcaacctggagtatatcccccgcacgcagcaggtcatttaccatatgtactatatgaccctacagctacagatgcaaaacaacaccacagacatggatatgaaaagcctgaagaattgtggacagccaaaagccgtgtgcacccattgtaa

SEQ ID NO: 4 - DNA, 1665 bp, synthetic construct
  misc_feature 1..1665: note = Construct B
  source 1..1665: mol_type = other DNA
atgacttcagttaattctgcagaagccagcactggtgcaggaggggggggcagtaatcctgtcaaaagcatgtggagtgagggggccacttttagtgccaactctgtgacttgtacattttctagacagtttttaattccatatgacccagagcaccattataaggtgttttctcccgcagcaagtagctgccacaatgccagtggaaaggaggcaaaggtttgcaccattagtcccataatgggatactcaaccccatggagatatttagattttaatgctttaaacttatttttttcacctttagagtttcagcacttaattgaaaattatggaagtatagctcctgatgctttaactgtaaccatatcagaaattgctgttaaggatgttacagacaaaactggagggggggtgcaggttactgacagcactacagggcgcctatgcatgttagtagaccatgaatacaagtacccatatgtgttagggcaaggtcaagatactttagccccagaacttcctatttgggtatactttccccctcaatatgcttacttaacagtaggagatgttaacacacaaggaatttctggagacagcaaaaaattagcaagtgaagaatcagcattttatgttttggaacacagttcttttcagcttttaggtacaggaggtacagcaactatgtcttataagtttcctccagtgcccccagaaaatttagagggctgcagtcaacacttttatgagatgtacaatcccttatacggatcccgcttaggggttcctgacacattaggaggtgacccaaaatttagatctttaacacatgaagaccatgcaattcagccccaaaacttcatgccagggccactagtaaactcagtgtctacaaaggagggagacagctctaatactggagctgggaaagccttaacaggccttagcacaggtacctctcaaaacactagaatatccttacgcccggggccagtgtctcagccgtaccaccactgggacacagataaatatgtcacaggaataaatgctatttctcatggtcagaccacttatggtaacgctgaagacaaagagtatcagcaaggagtgggtagatttccaaatgaaaaagaacagctaaaacagttacagggtttaaacatgcacacctactttcccaataaaggaacccagcaatggacagatcaaattgagcgccccctaatggtgggttctgtatggaacagaagagcccttcactatgaaagccagctgtggagtaaaattccaaatttagatgacagttttaaaactcagtttgcagccttaggaggatggggtttgcatcagccacctcctcaaatatttttaaaaatattaccacaaagtgggccaattggaggtattaaatcaatgggaattactaccttagttcagtatgccgtgggaattatgacagtaaccatgacatttaaattggggccccgtaaagctacgggacggtggaatcctcaacctggagtatatcccccgcacgcagcaggtcatttaccatatgtactatatgaccctacagctacagatgcaaaacaacaccacagacatggatatgaaaagcctgaagaattgtggacagccaaaagccgtgtgcacccattgtaa

SEQ ID NO: 5 - DNA, 1665 bp, synthetic construct
  misc_feature 1..1665: note = Construct C
  source 1..1665: mol_type = other DNA
atgacttcagttaattctgcagaagccagcactggtgcaggaggggggggcagtaatcctgtcaaaagcatgtggagtgagggggccacttttagtgccaactctgtgacttgtacattttctagacagtttttaattccatatgacccagagcaccattataaggtgttttctcccgcagcaagtagctgccacaatgccagtggaaaggaggcaaaggtttgcaccattagtcccataatgggatactcaaccccatggagatatttagattttaatgctttaaacttatttttttcacctttagagtttcagcacttaattgaaaattatggaagtatagctcctgatgctttaactgtaaccatatcagaaattgctgttaaggatgttacagacaaaactggagggggggtgcaggttactgacagcactacagggcgcctatgcatgttagtagaccatgaatacaagtacccatatgtgttagggcaaggtcaagatactttagccccagaacttcctatttgggtatactttccccctcaatatgcttacttaacagtaggagatgttaacacacaaggaatttctggagacagcaaaaaattagcaagtgaagaatcagcattttatgttttggaacacagttcttttcagcttttaggtacaggaggtacagcaactatgtcttataagtttcctccagtgcccccagaaaatttagagggctgcagtcaacacttttatgagatgtacaatcccttatacggatcccgcttaggggttcctgacacattaggaggtgacccaaaatttagatctttaacacatgaagaccatgcaattcagccccaaaacttcatgccagggccactagtaaactcagtgtctacaaaggagggagacagctctaatactggagctgggaaagccttaacaggccttagcacaggtacctctcaaaacactagaatatccttacgcccggggccagtgtctcagccgtaccaccactgggacacagataaatatgtcacaggaataaatgctatttctcatggtcagaccacttatggtaacgctgaagacaaagagtatcagcaaggagtgggtagatttccaaatgaaaaagaacagctaaaacagttacagggtttaaacatgcacacctactttcccaataaaggaacccagcaagctacagatcaaattgagcgccccctaatggtgggttctgtatggaacagaagagcccttcactatgaaagccagctgtggagtaaaattccaaatttagatgacagttttaaaactcagtttgcagccttaggaggatggggtttgcatcagccacctcctcaaatatttttaaaaatattaccacaaagtgggccaattggaggtattaaatcaatgggaattactaccttagttcagtatgccgtgggaattatgacagtaaccatgacatttaaattggggccccgtaaagctacgggacggtggaatcctcaacctggagtatatcccccgcacgcagcaggtcatttaccatatgtactatatgaccctacagctacagatgcaaaacaacaccacagacatggatatgaaaagcctgaagaattgtggacagccaaaagccgtgtgcacccattgtaa

SEQ ID NO: 6 - DNA, 1665 bp, synthetic construct
  misc_feature 1..1665: note = Construct D
  source 1..1665: mol_type = other DNA
atgacttcagttaattctgcagaagccagcactggtgcaggaggggggggcagtaatcctgtcaaaagcatgtggagtgagggggccacttttagtgccaactctgtgacttgtacattttctagacagtttttaattccatatgacccagagcaccattataaggtgttttctcccgcagcaagtagctgccacaatgccagtggaaaggaggcaaaggtttgcaccattagtcccataatgggatactcaaccccatggagatatttagattttaatgctttaaacttatttttttcacctttagagtttcagcacttaattgaaaattatggaagtatagctcctgatgctttaactgtaaccatatcagaaattgctgttaaggatgttacagacaaaactggagggggggtgcaggttactgacagcactacagggcgcctatgcatgttagtagaccatgaatacaagtacccatatgtgttagggcaaggtcaagatactttagccccagaacttcctatttgggtatactttccccctcaatatgcttacttaacagtaggagatgttaacacacaaggaatttctggagacagcaaaaaattagcaagtgaagaatcagcattttatgttttggaacacagttcttttcagcttttaggtacaggaggtacagcaactatgtcttataagtttcctccagtgcccccagaaaatttagagggctgcagtcaacacttttatgagatgtacaatcccttatacggatcccgcttaggggttcctgacacattaggaggtgacccaaaatttagatctttaacacatgaagaccatgcaattcagccccaaaacttcatgccagggccactagtaaactcagtgtctacaaaggagggagacagctctaatactggagctgggaaagccttaacaggccttagcacaggtacctctcaaaacactagaatatccttacgcccggggccagtgtctcagccgtaccaccactgggacacagataaatatgtcacaggaataaatgctatttctcatggtcagaccacttatggtaacgctgaagacaaagagtatgctgctggagtgggtagatttccaaatgaaaaagaacagctaaaacagttacagggtttaaacatgcacacctactttcccaataaaggaacccagcaatatacagatcaaattgagcgccccctaatggtgggttctgtatggaacagaagagcccttcactatgaaagccagctgtggagtaaaattccaaatttagatgacagttttaaaactcagtttgcagccttaggaggatggggtttgcatcagccacctcctcaaatatttttaaaaatattaccacaaagtgggccaattggaggtattaaatcaatgggaattactaccttagttcagtatgccgtgggaattatgacagtaaccatgacatttaaattggggccccgtaaagctacgggacggtggaatcctcaacctggagtatatcccccgcacgcagcaggtcatttaccatatgtactatatgaccctacagctacagatgcaaaacaacaccacagacatggatatgaaaagcctgaagaattgtggacagccaaaagccgtgtgcacccattgtaa

SEQ ID NO: 7 - DNA, 1665 bp, synthetic construct
  misc_feature 1..1665: note = Construct E
  source 1..1665: mol_type = other DNA
atgacttcagttaattctgcagaagccagcactggtgcaggaggggggggcagtaatcctgtcaaaagcatgtggagtgagggggccacttttagtgccaactctgtgacttgtacattttctagacagtttttaattccatatgacccagagcaccattataaggtgttttctcccgcagcaagtagctgccacaatgccagtggaaaggaggcaaaggtttgcaccattagtcccataatgggatactcaaccccatggagatatttagattttaatgctttaaacttatttttttcacctttagagtttcagcacttaattgaaaattatggaagtatagctcctgatgctttaactgtaaccatatcagaaattgctgttaaggatgttacagacaaaactggagggggggtgcaggttactgacagcactacagggcgcctatgcatgttagtagaccatgaatacaagtacccatatgtgttagggcaaggtcaagatactttagccccagaacttcctatttgggtatactttccccctcaatatgcttacttaacagtaggagatgttaacacacaaggaatttctggagacagcaaaaaattagcaagtgaagaatcagcattttatgttttggaacacagttcttttcagcttttaggtacaggaggtacagcaactatgtcttataagtttcctccagtgcccccagaaaatttagagggctgcagtcaacacttttatgagatgtacaatcccttatacggatcccgcttaggggttcctgacacattaggaggtgacccaaaatttagatctttaacacatgaagaccatgcaattcagccccaaaacttcatgccagggccactagtaaactcagtgtctacaaaggagggagacagctctaatactggagctgggaaagccttaacaggccttagcacaggtacctctcaaaacactagaatatccttacgcccggggccagtgtctcagccgtaccaccactgggacacagataaatatgtcacaggaataaatgctatttctcatggtcagaccacttatggtaacgctgaagacaaagagtataacaacggagtgggtagatttccaaatgaaaaagaacagctaaaacagttacagggtttaaacatgcacacctactttcccaataaaggaacccagcaatatacagatcaaattgagcgccccctaatggtgggttctgtatggaacagaagagcccttcactatgaaagccagctgtggagtaaaattccaaatttagatgacagttttaaaactcagtttgcagccttaggaggatggggtttgcatcagccacctcctcaaatatttttaaaaatattaccacaaagtgggccaattggaggtattaaatcaatgggaattactaccttagttcagtatgccgtgggaattatgacagtaaccatgacatttaaattggggccccgtaaagctacgggacggtggaatcctcaacctggagtatatcccccgcacgcagcaggtcatttaccatatgtactatatgaccctacagctacagatgcaaaacaacaccacagacatggatatgaaaagcctgaagaattgtggacagccaaaagccgtgtgcacccattgtaa

SEQ ID NO: 8 - DNA, 1665 bp, synthetic construct
  misc_feature 1..1665: note = Construct F
  source 1..1665: mol_type = other DNA
atgacttcagttaattctgcagaagccagcactggtgcaggaggggggggcagtaatcctgtcaaaagcatgtggagtgagggggccacttttagtgccaactctgtgacttgtacattttctagacagtttttaattccatatgacccagagcaccattataaggtgttttctcccgcagcaagtagctgccacaatgccagtggaaaggaggcaaaggtttgcaccattagtcccataatgggatactcaaccccatggagatatttagattttaatgctttaaacttatttttttcacctttagagtttcagcacttaattgaaaattatggaagtatagctcctgatgctttaactgtaaccatatcagaaattgctgttaaggatgttacagacaaaactggagggggggtgcaggttactgacagcactacagggcgcctatgcatgttagtagaccatgaatacaagtacccatatgtgttagggcaaggtcaagatactttagccccagaacttcctatttgggtatactttccccctcaatatgcttacttaacagtaggagatgttaacacacaaggaatttctggagacagcaaaaaattagcaagtgaagaatcagcattttatgttttggaacacagttcttttcagcttttaggtacaggaggtacagcaactatgtcttataagtttcctccagtgcccccagaaaatttagagggctgcagtcaacacttttatgagatgtacaatcccttatacggatcccgcttaggggttcctgacacattaggaggtgacccaaaatttagatctttaacacatgaagaccatgcaattcagccccaaaacttcatgccagggccactagtaaactcagtgtctacaaaggagggagacagctctaatactggagctgggaaagccttaacaggccttagcacaggtacctctcaaaacactagaatatccttacgcccggggccagtgtctcagccgtaccaccactgggacacagataaatatgtcacaggaataaatgctatttctcatggtcagaccacttatggtaacgctgaagacaaagagtatcagcaaggagtgggtagatttccaaatgaaaaagaacagctaaaacagttacagggtttaaacatgcacacctactttcccaataaaggaaccaacaactttacagataacattgagcgccccctaatggtgggttctgtatggaacagaagagcccttcactatgaaagccagctgtggagtaaaattccaaatttagatgacagttttaaaactcagtttgcagccttaggaggatggggtttgcatcagccacctcctcaaatatttttaaaaatattaccacaaagtgggccaattggaggtattaaatcaatgggaattactaccttagttcagtatgccgtgggaattatgacagtaaccatgacatttaaattggggccccgtaaagctacgggacggtggaatcctcaacctggagtatatcccccgcacgcagcaggtcatttaccatatgtactatatgaccctacagctacagatgcaaaacaacaccacagacatggatatgaaaagcctgaagaattgtggacagccaaaagccgtgtgcacccattgtaa

SEQ ID NO: 9 - DNA, 1665 bp, synthetic construct
  misc_feature 1..1665: note = Construct G
  source 1..1665: mol_type = other DNA
atgacttcagttaattctgcagaagccagcactggtgcaggaggggggggcagtaatcctgtcaaaagcatgtggagtgagggggccacttttagtgccaactctgtgacttgtacattttctagacagtttttaattccatatgacccagagcaccattataaggtgttttctcccgcagcaagtagctgccacaatgccagtggaaaggaggcaaaggtttgcaccattagtcccataatgggatactcaaccccatggagatatttagattttaatgctttaaacttatttttttcacctttagagtttcagcacttaattgaaaattatggaagtatagctcctgatgctttaactgtaaccatatcagaaattgctgttaaggatgttacagacaaaactggagggggggtgcaggttactgacagcactacagggcgcctatgcatgttagtagaccatgaatacaagtacccatatgtgttagggcaaggtcaagatactttagccccagaacttcctatttgggtatactttccccctcaatatgcttacttaacagtaggagatgttaacacacaaggaatttctggagacagcaaaaaattagcaagtgaagaatcagcattttatgttttggaacacagttcttttcagcttttaggtacaggaggtacagcaactatgtcttataagtttcctccagtgcccccagaaaatttagagggctgcagtcaacacttttatgagatgtacaatcccttatacggatcccgcttaggggttcctgacacattaggaggtgacccaaaatttagatctttaacacatgaagaccatgcaattcagccccaaaacttcatgccagggccactagtaaactcagtgtctacaaaggagggagacagctctaatactggagctgggaaagccttaacaggccttagcacaggtacctctcaaaacactagaatatccttacgcccggggccagtgtctcagccgtaccaccactgggacacagataaatatgtcacaggaataaatgctatttctcatggtcagaccacttatggtaacgctgaagacaaagagtatcagcaaggagtgggtagatttccaaatgaaaaagaacagctaaaacagttacagggtttaaacatgcacacctactttcccaataaaggaaccaacaactatacagataacattgagcgccccctaatggtgggttctgtatggaacagaagagcccttcactatgaaagccagctgtggagtaaaattccaaatttagatgacagttttaaaactcagtttgcagccttaggaggatggggtttgcatcagccacctcctcaaatatttttaaaaatattaccacaaagtgggccaattggaggtattaaatcaatgggaattactaccttagttcagtatgccgtgggaattatgacagtaaccatgacatttaaattggggccccgtaaagctacgggacggtggaatcctcaacctggagtatatcccccgcacgcagcaggtcatttaccatatgtactatatgaccctacagctacagatgcaaaacaacaccacagacatggatatgaaaagcctgaagaattgtggacagccaaaagccgtgtgcacccattgtaa

SEQ ID NO: 10 - DNA, 1665 bp, synthetic construct
  misc_feature 1..1665: note = Construct H
  source 1..1665: mol_type = other DNA
atgacttcagttaattctgcagaagccagcactggtgcaggaggggggggcagtaatcctgtcaaaagcatgtggagtgagggggccacttttagtgccaactctgtgacttgtacattttctagacagtttttaattccatatgacccagagcaccattataaggtgttttctcccgcagcaagtagctgccacaatgccagtggaaaggaggcaaaggtttgcaccattagtcccataatgggatactcaaccccatggagatatttagattttaatgctttaaacttatttttttcacctttagagtttcagcacttaattgaaaattatggaagtatagctcctgatgctttaactgtaaccatatcagaaattgctgttaaggatgttacagacaaaactggagggggggtgcaggttactgacagcactacagggcgcctatgcatgttagtagaccatgaatacaagtacccatatgtgttagggcaaggtcaagatactttagccccagaacttcctatttgggtatactttccccctcaatatgcttacttaacagtaggagatgttaacacacaaggaatttctggagacagcaaaaaattagcaagtgaagaatcagcattttatgttttggaacacagttcttttcagcttttaggtacaggaggtacagcaactatgtcttataagtttcctccagtgcccccagaaaatttagagggctgcagtcaacacttttatgagatgtacaatcccttatacggatcccgcttaggggttcctgacacattaggaggtgacccaaaatttagatctttaacacatgaagaccatgcaattcagccccaaaacttcatgccagggccactagtaaactcagtgtctacaaaggagggagacagctctaatactggagctgggaaagccttaacaggccttagcacaggtacctctcaaaacactagaatatccttacgcccggggccagtgtctcagccgtaccaccactgggacacagataaatatgtcacaggaataaatgctatttctcatggtcagaccacttatggtaacgctgaagacaaagagtatcagcaaggagtgggtagatttccaaatgaaaaagaacagctaaaacagttacagggtttaaacatgcacaccgcttttcccaataaaggaacccagcaatatacagatcaaattgagcgccccctaatggtgggttctgtatggaacagaagagcccttcactatgaaagccagctgtggagtaaaattccaaatttagatgacagttttaaaactcagtttgcagccttaggaggatggggtttgcatcagccacctcctcaaatatttttaaaaatattaccacaaagtgggccaattggaggtattaaatcaatgggaattactaccttagttcagtatgccgtgggaattatgacagtaaccatgacatttaaattggggccccgtaaagctacgggacggtggaatcctcaacctggagtatatcccccgcacgcagcaggtcatttaccatatgtactatatgaccctacagctacagatgcaaaacaacaccacagacatggatatgaaaagcctgaagaattgtggacagccaaaagccgtgtgcacccattgtaa

SEQ ID NO: 11 - DNA, 1665 bp, synthetic construct
  misc_feature 1..1665: note = Construct I
  source 1..1665: mol_type = other DNA
atgacttcagttaattctgcagaagccagcactggtgcaggaggggggggcagtaatcctgtcaaaagcatgtggagtgagggggccacttttagtgccaactctgtgacttgtacattttctagacagtttttaattccatatgacccagagcaccattataaggtgttttctcccgcagcaagtagctgccacaatgccagtggaaaggaggcaaaggtttgcaccattagtcccataatgggatactcaaccccatggagatatttagattttaatgctttaaacttatttttttcacctttagagtttcagcacttaattgaaaattatggaagtatagctcctgatgctttaactgtaaccatatcagaaattgctgttaaggatgttacagacaaaactggagggggggtgcaggttactgacagcactacagggcgcctatgcatgttagtagaccatgaatacaagtacccatatgtgttagggcaaggtcaagatactttagccccagaacttcctatttgggtatactttccccctcaatatgcttacttaacagtaggagatgttaacacacaaggaatttctggagacagcaaaaaattagcaagtgaagaatcagcattttatgttttggaacacagttcttttcagcttttaggtacaggaggtacagcaactatgtcttataagtttcctccagtgcccccagaaaatttagagggctgcagtcaacacttttatgagatgtacaatcccttatacggatcccgcttaggggttcctgacacattaggaggtgacccaaaatttagatctttaacacatgaagaccatgcaattcagccccaaaacttcatgccagggccactagtaaactcagtgtctacaaaggagggagacagctctaatactggagctgggaaagccttaacaggccttagcacaggtacctctcaaaacactagaatatccttacgcccggggccagtgtctcagccgtaccaccactgggacacagataaatatgtcacaggaataaatgctatttctcatggtcagaccacttatggtaacgctgaagacaaagagtatcagcaaggagtgggtagatttccaaatgaaaaagaacagctaaaacagttacagggtttaaacatgcacaccttttttcccaataaaggaacccagcaatatacagatcaaattgagcgccccctaatggtgggttctgtatggaacagaagagcccttcactatgaaagccagctgtggagtaaaattccaaatttagatgacagttttaaaactcagtttgcagccttaggaggatggggtttgcatcagccacctcctcaaatatttttaaaaatattaccacaaagtgggccaattggaggtattaaatcaatgggaattactaccttagttcagtatgccgtgggaattatgacagtaaccatgacatttaaattggggccccgtaaagctacgggacggtggaatcctcaacctggagtatatcccccgcacgcagcaggtcatttaccatatgtactatatgaccctacagctacagatgcaaaacaacaccacagacatggatatgaaaagcctgaagaattgtggacagccaaaagccgtgtgcacccattgtaa

SEQ ID NO: 12 - DNA, 1665 bp, synthetic construct; identical to SEQ ID NO: 8
  misc_feature 1..1665: note = Construct J
  source 1..1665: mol_type = other DNA

SEQ ID NO: 13 - DNA, 1665 bp, synthetic construct; identical to SEQ ID NO: 9
  misc_feature 1..1665: note = Construct K
  source 1..1665: mol_type = other DNA

SEQ ID NO: 14 - DNA, 1677 bp, synthetic construct
  misc_feature 1..1677: note = Construct L
  source 1..1677: mol_type = other DNA
atgacttcagttaattctgcagaagccagcactggtgcaggaggggggggcagtaatcctgtcaaaagcatgtggagtgagggggccacttttagtgccaactctgtgacttgtacattttctagacagtttttaattccatatgacccagagcaccattataaggtgttttctcccgcagcaagtagctgccacaatgccagtggaaaggaggcaaaggtttgcaccattagtcccataatgggatactcaaccccatggagatatttagattttaatgctttaaacttatttttttcacctttagagtttcagcacttaattgaaaattatggaagtatagctcctgatgctttaactgtaaccatatcagaaattgctgttaaggatgttacagacaaaactggagggggggtgcaggttactgacagcactacagggcgcctatgcatgttagtagaccatgaatacaagtacccatatgtgttagggcaaggtcaagatactttagccccagaacttcctatttgggtatactttccccctcaatatgcttacttaacagtaggagatgttaacacacaaggaatttctggagacagcaaaaaattagcaagtgaagaatcagcattttatgttttggaacacagttcttttcagcttttaggtacaggaggtacagcaactatgtcttataagtttcctccagtgcccccagaaaatttagagggctgcagtcaacacttttatgagatgtacaatcccttatacggatcccgcttaggggttcctgacacattaggaggtgacccaaaatttagatctttaacacatgaagaccatgcaattcagccccaaaacttcatgccagggccactagtaaactcagtgtctacaaaggagggagacagctctaatactggagctgggaaagccttaacaggccttagcacaggtacctctcaaaacactagaatatccttacgcccggggccagtgtctcagccgtaccaccactgggacacagataaatatgtcacaggaataaatgctatttctcatggtcagaccacttatggtaacgctgaagacaaagagtatcagcaaggagtgggtagatttccaaatgaaaaagaacagctaaaacagttacagggtttaaacatgcacacctactttcccaataaaggaacccagcaatatacagatcaagatccaattggtattgagcgccccctaatggtgggttctgtatggaacagaagagcccttcactatgaaagccagctgtggagtaaaattccaaatttagatgacagttttaaaactcagtttgcagccttaggaggatggggtttgcatcagccacctcctcaaatatttttaaaaatattaccacaaagtgggccaattggaggtattaaatcaatgggaattactaccttagttcagtatgccgtgggaattatgacagtaaccatgacatttaaattggggccccgtaaagctacgggacggtggaatcctcaacctggagtatatcccccgcacgcagcaggtcatttaccatatgtactatatgaccctacagctacagatgcaaaacaacaccacagacatggatatgaaaagcctgaagaattgtggacagccaaaagccgtgtgcacccattgtaa

SEQ ID NO: 15 - DNA, 1665 bp, synthetic construct
  misc_feature 1..1665: note = Construct M
  source 1..1665: mol_type = other DNA
atgacttcagttaattctgcagaagccagcactggtgcaggaggggggggcagtaatcctgtcaaaagcatgtggagtgagggggccacttttagtgccaactctgtgacttgtacattttctagacagtttttaattccatatgacccagagcaccattataaggtgttttctcccgcagcaagtagctgccacaatgccagtggaaaggaggcaaaggtttgcaccattagtcccataatgggatactcaaccccatggagatatttagattttaatgctttaaacttatttttttcacctttagagtttcagcacttaattgaaaattatggaagtatagctcctgatgctttaactgtaaccatatcagaaattgctgttaaggatgttacagacaaaactggagggggggtgcaggttactgacagcactacagggcgcctatgcatgttagtagaccatgaatacaagtacccatatgtgttagggcaaggtcaagatactttagccccagaacttcctatttgggtatactttccccctcaatatgcttacttaacagtaggagatgttaacacacaaggaatttctggagacagcaaaaaattagcaagtgaagaatcagcattttatgttttggaacacagttcttttcagcttttaggtacaggaggtacagcaactatgtcttataagtttcctccagtgcccccagaaaatttagagggctgcagtcaacacttttatgagatgtacaatcccttatacggatcccgcttaggggttcctgacacattaggaggtgacccaaaatttagatctttaacacatgaagaccatgcaattcagccccaaaacttcatgccagggccactagtaaactcagtgtctacaaaggagggagacagctctaatactggagctgggaaagccttaacaggccttagcacaggtacctctcaaaacactagaatatccttacgcccggggccagtgtctcagccgtaccaccactgggacacagataaatatgtcacaggaataaatgctatttctcatggtcagaccacttatggtaacgctgaagacaaagagtatcagcaaggagtgggtagatttccaaatgaaaaagaacagctaaaacagttacagggtttaaacatgcacacctactttcccaataaaggaaccgctgcttatacagatcaaattgagcgccccctaatggtgggttctgtatggaacagaagagcccttcactatgaaagccagctgtggagtaaaattccaaatttagatgacagttttaaaactcagtttgcagccttaggaggatggggtttgcatcagccacctcctcaaatatttttaaaaatattaccacaaagtgggccaattggaggtattaaatcaatgggaattactaccttagttcagtatgccgtgggaattatgacagtaaccatgacatttaaattggggccccgtaaagctacgggacggtggaatcctcaacctggagtatatcccccgcacgcagcaggtcatttaccatatgtactatatgaccctacagctacagatgcaaaacaacaccacagacatggatatgaaaagcctgaagaattgtggacagccaaaagccgtgtgcacccattgtaa

SEQ ID NO: 16 - DNA, 1665 bp, synthetic construct
  misc_feature 1..1665: note = Construct N
  source 1..1665: mol_type = other DNA
atgacttcagttaattctgcagaagccagcactggtgcaggaggggggggcagtaatcctgtcaaaagcatgtggagtgagggggccacttttagtgccaactctgtgacttgtacattttctagacagtttttaattccatatgacccagagcaccattataaggtgttttctcccgcagcaagtagctgccacaatgccagtggaaaggaggcaaaggtttgcaccattagtcccataatgggatactcaaccccatggagatatttagattttaatgctttaaacttatttttttcacctttagagtttcagcacttaattgaaaattatggaagtatagctcctgatgctttaactgtaaccatatcagaaattgctgttaaggatgttacagacaaaactggagggggggtgcaggttactgacagcactacagggcgcctatgcatgttagtagaccatgaatacaagtacccatatgtgttagggcaaggtcaagatactttagccccagaacttcctatttgggtatactttccccctcaatatgcttacttaacagtaggagatgttaacacacaaggaatttctggagacagcaaaaaattagcaagtgaagaatcagcattttatgttttggaacacagttcttttcagcttttaggtacaggaggtacagcaactatgtcttataagtttcctccagtgcccccagaaaatttagagggctgcagtcaacacttttatgagatgtacaatcccttatacggatcccgcttaggggttcctgacacattaggaggtgacccaaaatttagatctttaacacatgaagaccatgcaattcagccccaaaacttcatgccagggccactagtaaactcagtgtctacaaaggagggagacagctctaatactggagctgggaaagccttaacaggccttagcacaggtacctctcaaaacactagaatatccttacgcccggggccagtgtctcagccgtaccaccactgggacacagataaatatgtcacaggaataaatgctatttctcatggtcagaccacttatggtaacgctgaagacaaagagtatcagcaaggagtgggtagatttccaaatgaaaaagaacagctaaaacagttacagggtttaaacatgcacacctactttcccaataaaggaacccaacaaccagctgcacaaattgagcgccccctaatggtgggttctgtatggaacagaagagcccttcactatgaaagccagctgtggagtaaaattccaaatttagatgacagttttaaaactcagtttgcagccttaggaggatggggtttgcatcagccacctcctcaaatatttttaaaaatattaccacaaagtgggccaattggaggtattaaatcaatgggaattactaccttagttcagtatgccgtgggaattatgacagtaaccatgacatttaaattggggccccgtaaagctacgggacggtggaatcctcaacctggagtatatcccccgcacgcagcaggtcatttaccatatgtactatatgaccctacagctacagatgcaaaacaacaccacagacatggatatgaaaagcctgaagaattgtggacagccaaaagccgtgtgcacccattgtaa

SEQ ID NO: 17 - DNA, 1665 bp, synthetic construct
  misc_feature 1..1665: note = Construct O
  source 1..1665: mol_type = other DNA
atgacttcagttaattctgcagaagccagcactggtgcaggaggggggggcagtaatcctgtcaaaagcatgtggagtgagggggccacttttagtgccaactctgtgacttgtacattttctagacagtttttaattccatatgacccagagcaccattataaggtgttttctcccgcagcaagtagctgccacaatgccagtggaaaggaggcaaaggtttgcaccattagtcccataatgggatactcaaccccatggagatatttagattttaatgctttaaacttatttttttcacctttagagtttcagcacttaattgaaaattatggaagtatagctcctgatgctttaactgtaaccatatcagaaattgctgttaaggatgttacagacaaaactggagggggggtgcaggttactgacagcactacagggcgcctatgcatgttagtagaccatgaatacaagtacccatatgtgttagggcaaggtcaagatactttagccccagaacttcctatttgggtatactttccccctcaatatgcttacttaacagtaggagatgttaacacacaaggaatttctggagacagcaaaaaattagcaagtgaagaatcagcattttatgttttggaacacagttcttttcagcttttaggtacaggaggtacagcaactatgtcttataagtttcctccagtgcccccagaaaatttagagggctgcagtcaacacttttatgagatgtacaatcccttatacggatcccgcttaggggttcctgacacattaggaggtgacccaaaatttagatctttaacacatgaagaccatgcaattcagccccaaaacttcatgccagggccactagtaaactcagtgtctacaaaggagggagacagctctaatactggagctgggaaagccttaacaggccttagcacaggtacctctcaaaacactagaatatccttacgcccggggccagtgtctcagccgtaccaccactgggacacagataaatatgtcacaggaataaatgctatttctcatggtcagaccacttatggtaacgctgaagacaaagagtatcagcaaggagtgggtagatttccaaatgaaaaagaacagctaaaacagttacagggtttaaacatgcacacctactttcccaataaaggaaccaacaactggacagataccattgagcgccccctaatggtgggttctgtatggaacagaagagcccttcactatgaaagccagctgtggagtaaaattccaaatttagatgacagttttaaaactcagtttgcagccttaggaggatggggtttgcatcagccacctcctcaaatatttttaaaaatattaccacaaagtgggccaattggaggtattaaatcaatgggaattactaccttagttcagtatgccgtgggaattatgacagtaaccatgacatttaaattggggccccgtaaagctacgggacggtggaatcctcaacctggagtatatcccccgcacgcagcaggtcatttaccatatgtactatatgaccctacagctacagatgcaaaacaacaccacagacatggatatgaaaagcctgaagaattgtggacagccaaaagccgtgtgcacccattgtaa

SEQ ID NO: 18 - DNA, 1665 bp, synthetic construct
  misc_feature 1..1665: note = Construct P
  source 1..1665: mol_type = other DNA
atgacttcagttaattctgcagaagccagcactggtgcaggaggggggggcagtaatcctgtcaaaagcatgtggagtgagggggccacttttagtgccaactctgtgacttgtacattttctagacagtttttaattccatatgacccagagcaccattataaggtgttttctcccgcagcaagtagctgccacaatgccagtggaaaggaggcaaaggtttgcaccattagtcccataatgggatactcaaccccatggagatatttagattttaatgctttaaacttatttttttcacctttagagtttcagcacttaattgaaaattatggaagtatagctcctgatgctttaactgtaaccatatcagaaattgctgttaaggatgttacagacaaaactggagggggggtgcaggttactgacagcactacagggcgcctatgcatgttagtagaccatgaatacaagtacccatatgtgttagggcaaggtcaagatactttagccccagaacttcctatttgggtatactttccccctcaatatgcttacttaacagtaggagatgttaacacacaaggaatttctggagacagcaaaaaattagcaagtgaagaatcagcattttatgttttggaacacagttcttttcagcttttaggtacaggaggtacagcaactatgtcttataagtttcctccagtgcccccagaaaatttagagggctgcagtcaacacttttatgagatgtacaatcccttatacggatcccgcttaggggttcctgacacattaggaggtgacccaaaatttagatctttaacacatgaagaccatgcaattcagccccaaaacttcatgccagggccactagtaaactcagtgtctacaaaggagggagacagctctaatactggagctgggaaagccttaacaggccttagcacaggtacctctcaaaacactagaatatccttacgcccggggccagtgtctcagccgtaccaccactgggacacagataaatatgtcacaggaataaatgctatttctcatggtcagaccacttatggtaacgctgaagacaaagagtatcagcaaggagtgggtagatttccaaatgaaaaagaacagctaaaacagttacagggtttaaacatgcacaccgcttttcccaataaaggaaccaacaactggacagataccattgagcgccccctaatggtgggttctgtatggaacagaagagcccttcactatgaaagccagctgtggagtaaaattccaaatttagatgacagttttaaaactcagtttgcagccttaggaggatggggtttgcatcagccacctcctcaaatatttttaaaaatattaccacaaagtgggccaattggaggtattaaatcaatgggaattactaccttagttcagtatgccgtgggaattatgacagtaaccatgacatttaaattggggccccgtaaagctacgggacggtggaatcctcaacctggagtatatcccccgcacgcagcaggtcatttaccatatgtactatatgaccctacagctacagatgcaaaacaacaccacagacatggatatgaaaagcctgaagaattgtggacagccaaaagccgtgtgcacccattgtaa

SEQ ID NO: 19 - DNA, 1665 bp, synthetic construct
  misc_feature 1..1665: note = Construct Q
  source 1..1665: mol_type = other DNA
atgacttcagttaattctgcagaagccagcactggtgcaggaggggggggcagtaatcctgtcaaaagcatgtggagtgagggggccacttttagtgccaactctgtgacttgtacattttctagacagtttttaattccatatgacccagagcaccattataaggtgttttctcccgcagcaagtagctgccacaatgccagtggaaaggaggcaaaggtttgcaccattagtcccataatgggatactcaaccccatggagatatttagattttaatgctttaaacttatttttttcacctttagagtttcagcacttaattgaaaattatggaagtatagctcctgatgctttaactgtaaccatatcagaaattgctgttaaggatgttacagacaaaactggagggggggtgcaggttactgacagcactacagggcgcctatgcatgttagtagaccatgaatacaagtacccatatgtgttagggcaaggtcaagatactttagccccagaacttcctatttgggtatactttccccctcaatatgcttacttaacagtaggagatgttaacacacaaggaatttctggagacagcaaaaaattagcaagtgaagaatcagcattttatgttttggaacacagttcttttcagcttttaggtacaggaggtacagcaactatgtcttataagtttcctccagtgcccccagaaaatttagagggctgcagtcaacacttttatgagatgtacaatcccttatacggatcccgcttaggggttcctgacacattaggaggtgacccaaaatttagatctttaacacatgaagaccatgcaattcagccccaaaacttcatgccagggccactagtaaactcagtgtctacaaaggagggagacagctctaatactggagctgggaaagccttaacaggccttagcacaggtacctctcaaaacactagaatatccttacgcccggggccagtgtctcagccgtaccaccactgggacacagataaatatgtcacaggaataaatgctatttctcatggtcagaccacttatggtaacgctgaagacaaagagtatgctgctggagtgggtagatttccaaatgaaaaagaacagctaaaacagttacagggtttaaacatgcacacctactttcccaataaaggaacccagcaatttacagatcaaattgagcgccccctaatggtgggttctgtatggaacagaagagcccttcactatgaaagccagctgtggagtaaaattccaaatttagatgacagttttaaaactcagtttgcagccttaggaggatggggtttgcatcagccacctcctcaaatatttttaaaaatattaccacaaagtgggccaattggaggtattaaatcaatgggaattactaccttagttcagtatgccgtgggaattatgacagtaaccatgacatttaaattggggccccgtaaagctacgggacggtggaatcctcaacctggagtatatcccccgcacgcagcaggtcatttaccatatgtactatatgaccctacagctacagatgcaaaacaacaccacagacatggatatgaaaagcctgaagaattgtggacagccaaaagccgtgtgcacccattgtaa

SEQ ID NO: 20 - DNA, 1665 bp, synthetic construct
  misc_feature 1..1665: note = Construct R
  source 1..1665: mol_type = other DNA
atgacttcagttaattctgcagaagccagcactggtgcaggaggggggggcagtaatcctgtcaaaagcatgtggagtgagggggccacttttagtgccaactctgtgacttgtacattttctagacagtttttaattccatatgacccagagcaccattataaggtgttttctcccgcagcaagtagctgccacaatgccagtggaaaggaggcaaaggtttgcaccattagtcccataatgggatactcaaccccatggagatatttagattttaatgctttaaacttatttttttcacctttagagtttcagcacttaattgaaaattatggaagtatagctcctgatgctttaactgtaaccatatcagaaattgctgttaaggatgttacagacaaaactggagggggggtgcaggttactgacagcactacagggcgcctatgcatgttagtagaccatgaatacaagtacccatatgtgttagggcaaggtcaagatactttagccccagaacttcctatttgggtatactttccccctcaatatgcttacttaacagtaggagatgttaacacacaaggaatttctggagacagcaaaaaattagcaagtgaagaatcagcattttatgttttggaacacagttcttttcagcttttaggtacaggaggtacagcaactatgtcttataagtttcctccagtgcccccagaaaatttagagggctgcagtcaacacttttatgagatgtacaatcccttatacggatcccgcttaggggttcctgacacattaggaggtgacccaaaatttagatctttaacacatgaagaccatgcaattcagccccaaaacttcatgccagggccactagtaaactcagtgtctacaaaggagggagacagctctaatactggagctgggaaagccttaacaggccttagcacaggtacctctcaaaacactagaatatccttacgcccggggccagtgtctcagccgtaccaccactgggacacagataaatatgtcacaggaataaatgctatttctcatggtcagaccacttatggtaacgctgaagacaaagagtatgctgctggagtgggtagatttccaaatgaaaaagaacagctaaaacagttacagggtttaaacatgcacacctactttcccaataaaggaaccaacaactttacagataccattgagcgccccctaatggtgggttctgtatggaacagaagagcccttcactatgaaagccagctgtggagtaaaattccaaatttagatgacagttttaaaactcagtttgcagccttaggaggatggggtttgcatcagccacctcctcaaatatttttaaaaatattaccacaaagtgggccaattggaggtattaaatcaatgggaattactaccttagttcagtatgccgtgggaattatgacagtaaccatgacatttaaattggggccccgtaaagctacgggacggtggaatcctcaacctggagtatatcccccgcacgcagcaggtcatttaccatatgtactatatgaccctacagctacagatgcaaaacaacaccacagacatggatatgaaaagcctgaagaattgtggacagccaaaagccgtgtgcacccattgtaa

SEQ ID NO: 21 - DNA, 1665 bp, synthetic construct
  misc_feature 1..1665: note = Construct S
  source 1..1665: mol_type = other DNA
atgacttcagttaattctgcagaagccagcactggtgcaggaggggggggcagtaatcctgtcaaaagcatgtggagtgagggggccacttttagtgccaactctgtgacttgtacattttctagacagtttttaattccatatgacccagagcaccattataaggtgttttctcccgcagcaagtagctgccacaatgccagtggaaaggaggcaaaggtttgcaccattagtcccataatgggatactcaaccccatggagatatttagattttaatgctttaaacttatttttttcacctttagagtttcagcacttaattgaaaattatggaagtatagctcctgatgctttaactgtaaccatatcagaaattgctgttaaggatgttacagacaaaactggagggggggtgcaggttactgacagcactacagggcgcctatgcatgttagtagaccatgaatacaagtacccatatgtgttagggcaaggtcaagatactttagccccagaacttcctatttgggtatactttccccctcaatatgcttacttaacagtaggagatgttaacacacaaggaatttctggagacagcaaaaaattagcaagtgaagaatcagcattttatgttttggaacacagttcttttcagcttttaggtacaggaggtacagcaactatgtcttataagtttcctccagtgcccccagaaaatttagagggctgcagtcaacacttttatgagatgtacaatcccttatacggatcccgcttaggggttcctgacacattaggaggtgacccaaaatttagatctttaacacatgaagaccatgcaattcagccccaaaacttcatgccagggccactagtaaactcagtgtctacaaaggagggagacagctctaatactggagctgggaaagccttaacaggccttagcacaggtacctctcaaaacactagaatatccttacgcccggggccagtgtctcagccgtaccaccactgggacacagataaatatgtcacaggaataaatgctatttctcatggtcagaccacttatggtaacgctgaagacaaagagtatcagcaaggagtgggtagatttccaaatgaaaaagaacagctaaaacagttacagggtttaaacatgcacaccgcttttcccaataaaggaacccagcaatggacagatcaaattgagcgccccctaatggtgggttctgtatggaacagaagagcccttcactatgaaagccagctgtggagtaaaattccaaatttagatgacagttttaaaactcagtttgcagccttaggaggatggggtttgcatcagccacctcctcaaatatttttaaaaatattaccacaaagtgggccaattggaggtattaaatcaatgggaattactaccttagttcagtatgccgtgggaattatgacagtaaccatgacatttaaattggggccccgtaaagctacgggacggtggaatcctcaacctggagtatatcccccgcacgcagcaggtcatttaccatatgtactatatgaccctacagctacagatgcaaaacaacaccacagacatggatatgaaaagcctgaagaattgtggacagccaaaagccgtgtgcacccattgtaa

SEQ ID NO: 22 - DNA, 1665 bp, synthetic construct
  misc_feature 1..1665: note = Construct T
  source 1..1665: mol_type = other DNA
atgacttcagttaattctgcagaagccagcactggtgcaggaggggggggcagtaatcctgtcaaaagcatgtggagtgagggggccacttttagtgccaactctgtgacttgtacattttctagacagtttttaattccatatgacccagagcaccattataaggtgttttctcccgcagcaagtagctgccacaatgccagtggaaaggaggcaaaggtttgcaccattagtcccataatgggatactcaaccccatggagatatttagattttaatgctttaaacttatttttttcacctttagagtttcagcacttaattgaaaattatggaagtatagctcctgatgctttaactgtaaccatatcagaaattgctgttaaggatgttacagacaaaactggagggggggtgcaggttactgacagcactacagggcgcctatgcatgttagtagaccatgaatacaagtacccatatgtgttagggcaaggtcaagatactttagccccagaacttcctatttgggtatactttccccctcaatatgcttacttaacagtaggagatgttaacacacaaggaatttctggagacagcaaaaaattagcaagtgaagaatcagcattttatgttttggaacacagttcttttcagcttttaggtacaggaggtacagcaactatgtcttataagtttcctccagtgcccccagaaaatttagagggctgcagtcaacacttttatgagatgtacaatcccttatacggatcccgcttaggggttcctgacacattaggaggtgacccaaaatttagatctttaacacatgaagaccatgcaattcagccccaaaacttcatgccagggccactagtaaactcagtgtctacaaaggagggagacagctctaatactggagctgggaaagccttaacaggccttagcacaggtacctctcaaaacactagaatatccttacgcccggggccagtgtctcagccgtaccaccactgggacacagataaatatgtcacaggaataaatgctatttctcatggtcagaccacttatggtaacgctgaagacaaagagtatgctgctggagtgggtagatttccaaatgaaaaagaacagctaaaacagttacagggtttaaacatgcacaccgcttttcccaataaaggaaccaacaactggacagataccattgagcgccccctaatggtgggttctgtatggaacagaagagcccttcactatgaaagccagctgtggagtaaaattccaaatttagatgacagttttaaaactcagtttgcagccttaggaggatggggtttgcatcagccacctcctcaaatatttttaaaaatattaccacaaagtgggccaattggaggtattaaatcaatgggaattactaccttagttcagtatgccgtgggaattatgacagtaaccatgacatttaaattggggccccgtaaagctacgggacggtggaatcctcaacctggagtatatcccccgcacgcagcaggtcatttaccatatgtactatatgaccctacagctacagatgcaaaacaacaccacagacatggatatgaaaagcctgaagaattgtggacagccaaaagccgtgtgcacccattgtaa

SEQ ID NO: 23 - DNA, 1665 bp, synthetic construct
  misc_feature 1..1665: note = Construct U
  source 1..1665: mol_type = other DNA
atgacttcagttaattctgcagaagccagcactggtgcaggaggggggggcagtaatcctgtcaaaagcatgtggagtgagggggccacttttagtgccaactctgtgacttgtacattttctagacagtttttaattccatatgacccagagcaccattataaggtgttttctcccgcagcaagtagctgccacaatgccagtggaaaggaggcaaaggtttgcaccattagtcccataatgggatactcaaccccatggagatatttagattttaatgctttaaacttatttttttcacctttagagtttcagcacttaattgaaaattatggaagtatagctcctgatgctttaactgtaaccatatcagaaattgctgttaaggatgttacagacaaaactggagggggggtgcaggttactgacagcactacagggcgcctatgcatgttagtagaccatgaatacaagtacccatatgtgttagggcaaggtcaagatactttagccccagaacttcctatttgggtatactttccccctcaatatgcttacttaacagtaggagatgttaacacacaaggaatttctggagacagcaaaaaattagcaagtgaagaatcagcattttatgttttggaacacagttcttttcagcttttaggtacaggaggtacagcaactatgtcttataagtttcctccagtgcccccagaaaatttagagggctgcagtcaacacttttatgagatgtacaatcccttatacggatcccgcttaggggttcctgacacattaggaggtgacccaaaatttagatctttaacacatgaagaccatgcaattcagccccaaaacttcatgccagggccactagtaaactcagtgtctacaaaggagggagacagctctaatactggagctgggaaagccttaacaggccttagcacaggtacctctcaaaacactagaatatccttacgcccggggccagtgtctcagccgtaccaccactgggacacagataaatatgtcacaggaataaatgctatttctcatggtcagaccacttatggtaacgctgaagacaaagagtatgctgctggagtgggtagatttccaaatgaaaaagaacagctaaaacagttacagggtttaaacatgcacaccgcttttcccaataaaggaacccagcaatttacagatcaaattgagcgccccctaatggtgggttctgtatggaacagaagagcccttcactatgaaagccagctgtggagtaaaattccaaatttagatgacagttttaaaactcagtttgcagccttaggaggatggggtttgcatcagccacctcctcaaatatttttaaaaatattaccacaaagtgggccaattggaggtattaaatcaatgggaattactaccttagttcagtatgccgtgggaattatgacagtaaccatgacatttaaattggggccccgtaaagctacgggacggtggaatcctcaacctggagtatatcccccgcacgcagcaggtcatttaccatatgtactatatgaccctacagctacagatgcaaaacaacaccacagacatggatatgaaaagcctgaagaattgtggacagccaaaagccgtgtgcacccattgtaa

SEQ ID NO: 24 - DNA, 1665 bp, synthetic construct
  misc_feature 1..1665: note = Construct V
  source 1..1665: mol_type = other DNA
atgacttcagttaattctgcagaagccagcactggtgcaggaggggggggcagtaatcctgtcaaaagcatgtggagtgagggggccacttttagtgccaactctgtgacttgtacattttctagacagtttttaattccatatgacccagagcaccattataaggtgttttctcccgcagcaagtagctgccacaatgccagtggaaaggaggcaaaggtttgcaccattagtcccataatgggatactcaaccccatggagatatttagattttaatgctttaaacttatttttttcacctttagagtttcagcacttaattgaaaattatggaagtatagctcctgatgctttaactgtaaccatatcagaaattgctgttaaggatgttacagacaaaactggagggggggtgcaggttactgacagcactacagggcgcctatgcatgttagtagaccatgaatacaagtacccatatgtgttagggcaaggtcaagatactttagccccagaacttcctatttgggtatactttccccctcaatatgcttacttaacagtaggagatgttaacacacaaggaatttctggagacagcaaaaaattagcaagtgaagaatcagcattttatgttttggaacacagttcttttcagcttttaggtacaggaggtacagcaactatgtcttataagtttcctccagtgcccccagaaaatttagagggctgcagtcaacacttttatgagatgtacaatcccttatacggatcccgcttaggggttcctgacacattaggaggtgacccaaaatttagatctttaacacatgaagaccatgcaattcagccccaaaacttcatgccagggccactagtaaactcagtgtctacaaaggagggagacagctctaatactggagctgggaaagccttaacaggccttagcacaggtacctctcaaaacactagaatatccttacgcccggggccagtgtctcagccgtaccaccactgggacacagataaatatgtcacaggaataaatgctatttctcatggtcagaccacttatggtaacgctgaagacaaagagtatcagcaaggagtgggtagatttccaaatgaaaaagaacagctaaaacagttacagggtttaaacatgcacaccgcttttcccaataaaggaacccagcaatttacagatcaaattgagcgccccctaatggtgggttctgtatggaacagaagagcccttcactatgaaagccagctgtggagtaaaattccaaatttagatgacagttttaaaactcagtttgcagccttaggaggatggggtttgcatcagccacctcctcaaatatttttaaaaatattaccacaaagtgggccaattggaggtattaaatcaatgggaattactaccttagttcagtatgccgtgggaattatgacagtaaccatgacatttaaattggggccccgtaaagctacgggacggtggaatcctcaacctggagtatatcccccgcacgcagcaggtcatttaccatatgtactatatgaccctacagctacagatgcaaaacaacaccacagacatggatatgaaaagcctgaagaattgtggacagccaaaagccgtgtgcacccattgtaa

SEQ ID NO: 25 - DNA, 1665 bp, synthetic construct
  misc_feature 1..1665: note = Construct W
  source 1..1665: mol_type = other DNA
atgacttcagttaattctgcagaagccagcactggtgcaggaggggggggcagtaatcctgtcaaaagcatgtggagtgagggggccacttttagtgccaactctgtgacttgtacattttctagacagtttttaattccatatgacccagagcaccattataaggtgttttctcccgcagcaagtagctgccacaatgccagtggaaaggaggcaaaggtttgcaccattagtcccataatgggatactcaaccccatggagatatttagattttaatgctttaaacttatttttttcacctttagagtttcagcacttaattgaaaattatggaagtatagctcctgatgctttaactgtaaccatatcagaaattgctgttaaggatgttacagacaaaactggagggggggtgcaggttactgacagcactacagggcgcctatgcatgttagtagaccatgaatacaagtacccatatgtgttagggcaaggtcaagatactttagccccagaacttcctatttgggtatactttccccctcaatatgcttacttaacagtaggagatgttaacacacaaggaatttctggagacagcaaaaaattagcaagtgaagaatcagcattttatgttttggaacacagttcttttcagcttttaggtacaggaggtacagcaactatgtcttataagtttcctccagtgcccccagaaaatttagagggctgcagtcaacacttttatgagatgtacaatcccttatacggatcccgcttaggggttcctgacacattaggaggtgacccaaaatttagatctttaacacatgaagaccatgcaattcagccccaaaacttcatgccagggccactagtaaactcagtgtctacaaaggagggagacagctctaatactggagctgggaaagccttaacaggccttagcacaggtacctctcaaaacactagaatatccttacgcccggggccagtgtctcagccgtaccaccactgggacacagataaatatgtcacaggaataaatgctatttctcatggtcagaccacttatggtaacgctgaagacaaagagtatgctgctggagtgggtagatttccaaatgaaaaagaacagctaaaacagttacagggtttaaacatgcacaccgcttttcccaataaaggaacccagcaatggacagatcaaattgagcgccccctaatggtgggttctgtatggaacagaagagcccttcactatgaaagccagctgtggagtaaaattccaaatttagatgacagttttaaaactcagtttgcagccttaggaggatggggtttgcatcagccacctcctcaaatatttttaaaaatattaccacaaagtgggccaattggaggtattaaatcaatgggaattactaccttagttcagtatgccgtgggaattatgacagtaaccatgacatttaaattggggccccgtaaagctacgggacggtggaatcctcaacctggagtatatcccccgcacgcagcaggtcatttaccatatgtactatatgaccctacagctacagatgcaaaacaacaccacagacatggatatgaaaagcctgaagaattgtggacagccaaaagccgtgtgcacccattgtaa

SEQ ID NO: 26 - DNA, 1665 bp, synthetic construct
  misc_feature 1..1665: note = Construct X
  source 1..1665: mol_type = other DNA
atgacttcagttaattctgcagaagccagcactggtgcaggaggggggggcagtaatcctgtcaaaagcatgtggagtgagggggccacttttagtgccaactctgtgacttgtacattttctagacagtttttaattccatatgacccagagcaccattataaggtgttttctcccgcagcaagtagctgccacaatgccagtggaaaggaggcaaaggtttgcaccattagtcccataatgggatactcaaccccatggagatatttagattttaatgctttaaacttatttttttcacctttagagtttcagcacttaattgaaaattatggaagtatagctcctgatgctttaactgtaaccatatcagaaattgctgttaaggatgttacagacaaaactggagggggggtgcaggttactgacagcactacagggcgcctatgcatgttagtagaccatgaatacaagtacccatatgtgttagggcaaggtcaagatactttagccccagaacttcctatttgggtatactttccccctcaatatgcttacttaacagtaggagatgttaacacacaaggaatttctggagacagcaaaaaattagcaagtgaagaatcagcattttatgttttggaacacagttcttttcagcttttaggtacaggaggtacagcaactatgtcttataagtttcctccagtgcccccagaaaatttagagggctgcagtcaacacttttatgagatgtacaatcccttatacggatcccgcttaggggttcctgacacattaggaggtgacccaaaatttagatctttaacacatgaagaccatgcaattcagccccaaaacttcatgccagggccactagtaaactcagtgtctacaaaggagggagacagctctaatactggagctgggaaagccttaacaggccttagcacaggtacctctcaaaacactagaatatccttacgcccggggccagtgtctcagccgtaccaccactgggacacagataaatatgtcacaggaataaatgctatttctcatggtcagaccacttatggtaacgctgaagacaaagagtatgctgctggagtgggtagatttccaaatgaaaaagaacagctaaaacagttacagggtttaaacatgcacaccgcttttcccaataaaggaacccagcaatatacagatcaaattgagcgccccctaatggtgggttctgtatggaacagaagagcccttcactatgaaagccagctgtggagtaaaattccaaatttagatgacagttttaaaactcagtttgcagccttaggaggatggggtttgcatcagccacctcctcaaatatttttaaaaatattaccacaaagtgggccaattggaggtattaaatcaatgggaattactaccttagttcagtatgccgtgggaattatgacagtaaccatgacatttaaattggggccccgtaaagctacgggacggtggaatcctcaacctggagtatatcccccgcacgcagcaggtcatttaccatatgtactatatgaccctacagctacagatgcaaaacaacaccacagacatggatatgaaaagcctgaagaattgtggacagccaaaagccgtgtgcacccattgtaa

SEQ ID NO: 27 - DNA, 31 bp, synthetic construct
  misc_feature 1..31: note = Wild type P1
  source 1..31: mol_type = other DNA
atgatggaattcatgacttcagttaattctg

SEQ ID NO: 28 - DNA, 35 bp, synthetic construct
  misc_feature 1..35: note = wild type P2
  source 1..35: mol_type = other DNA
atgatgctcgagaagcttacaatgggtgcacacgg

SEQ ID NO: 29 - DNA, 30 bp, synthetic construct
  misc_feature 1..30: note = Construct A P1
  source 1..30: mol_type = other DNA
ggggcgctcaatttgatctgtaaattgctg

SEQ ID NO: 30 - DNA, 30 bp, synthetic construct
  misc_feature 1..30: note = Construct A P2
  source 1..30: mol_type = other DNA
cccaataaaggaacccagcaatttacagat

SEQ ID NO: 31 - DNA, 30 bp, synthetic construct
  misc_feature 1..30: note = Construct B P1
  source 1..30: mol_type = other DNA
ggggcgctcaatttgatctgtccattgctg

SEQ ID NO: 32 - DNA, 30 bp, synthetic construct
  misc_feature 1..30: note = Construct B P2
  source 1..30: mol_type = other DNA
cccaataaaggaacccagcaatggacagat

SEQ ID NO: 33 - DNA, 30 bp, synthetic construct
  misc_feature 1..30: note = Construct C P1
  source 1..30: mol_type = other DNA
ggggcgctcaatttgatctgtagcttgctg

SEQ ID NO: 34 - DNA, 30 bp, synthetic construct
  misc_feature 1..30: note = Construct C P2
  source 1..30: mol_type = other DNA
cccaataaaggaacccagcaagctacagat

SEQ ID NO: 35 - DNA, 29 bp, synthetic construct
  misc_feature 1..29: note = Construct D P1
  source 1..29: mol_type = other DNA
ggaaatctacccactccagcagcatactc

SEQ ID NO: 36 - DNA, 30 bp, synthetic construct
  misc_feature 1..30: note = Construct D P2
  source 1..30: mol_type = other DNA
gctgaagacaaagagtatgctgctggagtg

SEQ ID NO: 37 - DNA, 29 bp, synthetic construct
  misc_feature 1..29: note = Construct E P1
  source 1..29: mol_type = other DNA
ggaaatctacccactccgttgttatactc

SEQ ID NO: 38 - DNA, 30 bp, synthetic construct
  misc_feature 1..30: note = Construct E P2
  source 1..30: mol_type = other DNA
gctgaagacaaagagtataacaacggagtg

SEQ ID NO: 39 - DNA, 47 bp, synthetic construct
  misc_feature 1..47: note = Construct F P1
  source 1..47: mol_type = other DNA
cccaccattagggggcgctcaatggtatctgtaaagttgttggttcc

SEQ ID NO: 40 - DNA, 51 bp, synthetic construct
  misc_feature 1..51: note = Construct F P2
  source 1..51: mol_type = other DNA
cacacctactttcccaataaaggaaccaacaactttacagataccattgag

SEQ ID NO: 41 - DNA, 47 bp, synthetic construct
  misc_feature 1..47: note = Construct G P1
  source 1..47: mol_type = other DNA
cccaccattagggggcgctcaatggtatctgtatagttgttggttcc

SEQ ID NO: 42 - DNA, 51 bp, synthetic construct
  misc_feature 1..51: note = Construct G P2
  source 1..51: mol_type = other DNA
cacacctactttcccaataaaggaaccaacaactatacagataccattgag

SEQ ID NO: 43 - DNA, 30 bp, synthetic construct
  misc_feature 1..30: note = Construct H P1
  source 1..30: mol_type = other DNA
ctgggttcctttattgggaaaagcggtgtg

SEQ ID NO: 44 - DNA, 27 bp, synthetic construct
  misc_feature 1..27: note = Construct H P2
  source 1..27: mol_type = other DNA
ggtttaaacatgcacaccgcttttccc

SEQ ID NO: 45 - DNA, 30 bp, synthetic construct
  misc_feature 1..30: note = Construct I P1
  source 1..30: mol_type = other DNA
ctgggttcctttattgggaaaaaaggtgtg

SEQ ID NO: 46 - DNA, 27 bp, synthetic construct
  misc_feature 1..27: note = Construct I P2
  source 1..27: mol_type = other DNA
ggtttaaacatgcacaccttttttccc

SEQ ID NO: 47 - DNA, 47 bp, synthetic construct
  misc_feature 1..47: note = Construct J P1
  source 1..47: mol_type = other DNA
cccaccattagggggcgctcaatgttatctgtaaagttgttggttcc

SEQ ID NO: 48 - DNA, 51 bp, synthetic construct
  misc_feature 1..51: note = Construct J P2
  source 1..51: mol_type = other DNA
cacacctactttcccaataaaggaaccaacaactttacagataacattgag

SEQ ID NO: 49 - DNA, 47 bp, synthetic construct
  misc_feature 1..47: note = Construct K P1
  source 1..47: mol_type = other DNA
cccaccattagggggcgctcaatgttatctgtatagttgttggttcc

SEQ ID NO: 50 - DNA, 51 bp, synthetic construct
  misc_feature 1..51: note = Construct K P2
  source 1..51: mol_type = other DNA
cacacctactttcccaataaaggaaccaacaactatacagataacattgag

SEQ ID NO: 51 - DNA, 41 bp, synthetic construct
  misc_feature 1..41: note = Construct L P1
  source 1..41: mol_type = other DNA
cccaccattagggggcgctcaataccaattggatcttgatc

SEQ ID NO: 52 - DNA, 36 bp, synthetic construct
  misc_feature 1..36: note = Construct L P2
  source 1..36: mol_type = other DNA
cagcaatatacagatcaagatccaattggtattgag

SEQ ID NO: 53 - DNA, 28 bp, synthetic construct
  misc_feature 1..28: note = Construct M P1
  source 1..28: mol_type = other DNA
ggcgctcaatttgatctgtataagcagc

SEQ ID NO: 54 - DNA, 30 bp, synthetic construct
  misc_feature 1..30: note = Construct M P2
  source 1..30: mol_type = other DNA
acctactttcccaataaaggaaccgctgct

SEQ ID NO: 55 - DNA, 42 bp, synthetic construct
  misc_feature 1..42: note = Construct N P1
  source 1..42: mol_type = other DNA
acccaccattagggggcgctcaatagctgcagctggttgttg

SEQ ID NO: 56 - DNA, 39 bp, synthetic construct
  misc_feature 1..39: note = Construct N P2
  source 1..39: mol_type = other DNA
acctactttcccaataaaggaacccaacaaccagctgca

SEQ ID NO: 57 - DNA, 47 bp, synthetic construct
  misc_feature 1..47: note = Construct O P1
  source 1..47: mol_type = other DNA
cccaccattagggggcgctcaatggtatctgtccagttgttggttcc

SEQ ID NO: 58 - DNA, 51 bp, synthetic construct
  misc_feature 1..51: note = Construct O P2
  source 1..51: mol_type = other DNA
cacacctactttcccaataaaggaaccaacaactggacagataccattgag

SEQ ID NO: 59 - DNA, 47 bp, synthetic construct; identical to SEQ ID NO: 57
  misc_feature 1..47: note = Construct P P1
  source 1..47: mol_type = other DNA

SEQ ID NO: 60 - DNA, 51 bp, synthetic construct; identical to SEQ ID NO: 58
  misc_feature 1..51: note = Construct P P2
  source 1..51: mol_type = other DNA

SEQ ID NO: 61 - DNA, 29 bp, synthetic construct
  misc_feature 1..29: note = Construct Q P1
  source 1..29: mol_type = other DNA
ggaaatctacccactccagcagcatactc

SEQ ID NO: 62 - DNA, 30 bp, synthetic construct; identical to SEQ ID NO: 36
  misc_feature 1..30: note = Construct Q P2
  source 1..30: mol_type = other DNA

SEQ ID NO: 63 - DNA, 29 bp, synthetic construct
  misc_feature 1..29: note = Construct R P1
  source 1..29: mol_type = other DNA
ggaaatctacccactccagcagcatactc

SEQ ID NO: 64 - DNA, 30 bp, synthetic construct; identical to SEQ ID NO: 36
  misc_feature 1..30: note = Construct R P2
  source 1..30: mol_type = other DNA

SEQ ID NO: 65 - DNA, 30 bp, synthetic construct; identical to SEQ ID NO: 43
  misc_feature 1..30: note = Construct S P1
  source 1..30: mol_type = other DNA

SEQ ID NO: 66 - DNA, 27 bp, synthetic construct
  misc_feature 1..27: note = Construct S P2
  source 1..27: mol_type = other DNA
ggtttaaacatgcacaccgcttttccc

SEQ ID NO: 67 - DNA, 29 bp, synthetic construct
  misc_feature 1..29: note = Construct T P1
  source 1..29: mol_type = other DNA
ggaaatctacccactccagcagcatactc

SEQ ID NO: 68 - DNA, 30 bp, synthetic construct; identical to SEQ ID NO: 36
  misc_feature 1..30: note = Construct T P2
  source 1..30: mol_type = other DNA

SEQ ID NO: 69 - DNA, 30 bp, synthetic construct; identical to SEQ ID NO: 43
  misc_feature 1..30: note = Construct U P1
  source 1..30: mol_type = other DNA

SEQ ID NO: 70 - DNA, 27 bp, synthetic construct
  misc_feature 1..27: note = Construct U P2
  source 1..27: mol_type = other DNA
ggtttaaacatgcacaccgcttttccc

SEQ ID NO: 71 - DNA, 30 bp, synthetic construct; identical to SEQ ID NO: 43
  misc_feature 1..30: note = Construct V P1
  source 1..30: mol_type = other DNA

SEQ ID NO: 72 - DNA, 27 bp, synthetic construct
  misc_feature 1..27: note = Construct V P2
  source 1..27: mol_type = other DNA
ggtttaaacatgcacaccgcttttccc

SEQ ID NO: 73 - DNA, 30 bp, synthetic construct; identical to SEQ ID NO: 43
  misc_feature 1..30: note = Construct W P1
  source 1..30: mol_type = other DNA

SEQ ID NO: 74 - DNA, 27 bp, synthetic construct
  misc_feature 1..27: note = Construct W P2
  source 1..27: mol_type = other DNA
ggtttaaacatgcacaccgcttttccc

SEQ ID NO: 75 - DNA, 29 bp, synthetic construct
  misc_feature 1..29: note = Construct X P1
  source 1..29: mol_type = other DNA
ggaaatctacccactccagcagcatactc

SEQ ID NO: 76 - DNA, 30 bp, synthetic construct; identical to SEQ ID NO: 36
  misc_feature 1..30: note = Construct X P2
  source 1..30: mol_type = other DNA